European Patent Specification EP 3 925 969 B1, published September 3, 2025. Title: PEPTIDE COMPOUNDS AND PEPTIDE CONJUGATES FOR THE TREATMENT OF CANCER THROUGH RECEPTOR MEDIATED CHEMOTHERAPY. Applicant: TRANSFERT PLUS, S.E.C. Application EP 21174271.3. The sequence listing filed with the application follows.

SEQUENCE LISTING (23 sequences)

SEQ ID NO: 1 - protein, 22 aa, Artificial Sequence
  Synthetic Construct
  MISC_FEATURE (1)..(5): Xaa can be any amino acid
  MISC_FEATURE (8)..(8): Xaa can be any amino acid
  MISC_FEATURE (14)..(14): Xaa can be any amino acid
  MISC_FEATURE (16)..(16): Xaa can be any amino acid
XXXXXGVXAKAGVXNXFKSESY

SEQ ID NO: 2 - protein, 23 aa, Artificial Sequence
  Synthetic Construct
  MISC_FEATURE (1)..(6): Xaa can be any amino acid and can be either present or absent
  MISC_FEATURE (9)..(9): Xaa can be any amino acid
  MISC_FEATURE (15)..(15): Xaa can be any amino acid
  MISC_FEATURE (17)..(17): Xaa can be any amino acid
XXXXXXGVXAKAGVXNXFKSESY

SEQ ID NO: 3 - protein, 24 aa, Artificial Sequence
  Synthetic Construct
  MISC_FEATURE (3)..(3): Xaa can be any amino acid
  MISC_FEATURE (7)..(7): Xaa can be any amino acid
  MISC_FEATURE (13)..(13): Xaa can be any amino acid
  MISC_FEATURE (22)..(23): Xaa can be either Gln, Pro, Tyr, Ile or Leu
YKXLRRXAPRWDXPLRDPALRXXL

SEQ ID NO: 4 - protein, 23 aa, Artificial Sequence
  Synthetic Construct
  MISC_FEATURE (3)..(3): Xaa can be any amino acid
  MISC_FEATURE (7)..(12): Xaa can be any amino acid and can be either present or absent
  MISC_FEATURE (21)..(22): Xaa can be either Gln, Pro, Tyr, Ile or Leu
YKXLRRXXXXXXPLRDPALRXXL

SEQ ID NO: 5 - protein, 22 aa, Artificial Sequence
  Synthetic Construct
IKLSGGVQAKAGVINMDKSESM

SEQ ID NO: 6 - protein, 22 aa, Artificial Sequence
  Synthetic Construct
IKLSGGVQAKAGVINMFKSESY

SEQ ID NO: 7 - protein, 23 aa, Artificial Sequence
  Synthetic Construct
IKLSGGVQAKAGVINMFKSESYK

SEQ ID NO: 8 - protein, 17 aa, Artificial Sequence
  Synthetic Construct
GVQAKAGVINMFKSESY

SEQ ID NO: 9 - protein, 17 aa, Artificial Sequence
  Synthetic Construct
GVRAKAGVRNMFKSESY

SEQ ID NO: 10 - protein, 17 aa, Artificial Sequence
  Synthetic Construct
  MISC_FEATURE (11)..(11): Xaa is Nle
GVRAKAGVRNXFKSESY

SEQ ID NO: 11 - protein, 24 aa, Artificial Sequence
  Synthetic Construct
YKSLRRKAPRWDAPLRDPALRQLL

SEQ ID NO: 12 - protein, 24 aa, Artificial Sequence
  Synthetic Construct
YKSLRRKAPRWDAYLRDPALRQLL

SEQ ID NO: 13 - protein, 24 aa, Artificial Sequence
  Synthetic Construct
YKSLRRKAPRWDAYLRDPALRPLL

SEQ ID NO: 14 - protein, 17 aa, Artificial Sequence
  Synthetic Construct
  MOD_RES (1)..(1): ACETYLATION
GVRAKAGVRNMFKSESY

SEQ ID NO: 15 - protein, 17 aa, Artificial Sequence
  Synthetic Construct
  MOD_RES (1)..(1): ACETYLATION
  MISC_FEATURE (11)..(11): Xaa is Nle
GVRAKAGVRNXFKSESY

SEQ ID NO: 16 - protein, 24 aa, Artificial Sequence
  Synthetic Construct
  MOD_RES (1)..(1): ACETYLATION
YKSLRRKAPRWDAPLRDPALRQLL

SEQ ID NO: 17 - protein, 24 aa, Artificial Sequence
  Synthetic Construct
  MOD_RES (1)..(1): ACETYLATION
YKSLRRKAPRWDAYLRDPALRQLL

SEQ ID NO: 18 - protein, 24 aa, Artificial Sequence
  Synthetic Construct
  MOD_RES (1)..(1): ACETYLATION
YKSLRRKAPRWDAYLRDPALRPLL

SEQ ID NO: 19 - protein, 23 aa, Homo sapiens
KCLRREAPRWDAPLRDPALRQLL

SEQ ID NO: 20 - protein, 23 aa, Rattus norvegicus
KCLRKKTPRWDILLRDPAPRPLL

SEQ ID NO: 21 - protein, 23 aa, Mus musculus
KCLRKKIPRWDMFLRDPVPRPLL

SEQ ID NO: 22 - protein, 13 aa, Homo sapiens
  MISC_FEATURE (1)..(1): Xaa can be any amino acid
XLYENKPRRPYIL

SEQ ID NO: 23 - protein, 23 aa, Artificial Sequence
  Synthetic Construct
IKLSGGVQAKAGVINMDKSESMY